European Patent Application EP 4 349 869 A1, published April 10, 2024. Title: VACCINE COMPOSITION FOR TREATING OR PREVENTING VIRAL DISEASES. Applicant: LEMONEX INC. The sequence listing filed with the application follows.

SEQUENCE LISTING (12 sequences)

SEQ ID NO: 1 - DNA, 81 bp, Artificial Sequence
  stabilization sequence
ggctacatccctgaagcgcctagagacggccagtgctacgtgagatgcgacggcgaatgggtgctgctgtccactttcctg

SEQ ID NO: 2 - DNA, 699 bp, Artificial Sequence
  COVID-19 Receptor binding domain coding sequence
agagtccaaccaacagaatctattgttagatttcctaatattacaaacttgtgcccttttggtgaagtttttaacgccaccagatttgcatctgtttatgcttggaacaggaagagaatcagcaactgtgttgctgattattctgtcctatataattccgcatcattttccacttttaagtgttatggagtgtctcctactaaattaaatgatctctgctttactaatgtctatgcagattcatttgtaattagaggtgatgaagtcagacaaatcgctccagggcaaactggaaagattgctgattataattataaattaccagatgattttacaggctgcgttatagcttggaattctaacaatcttgattctaaggttggtggtaattataattaccggtatagattgtttaggaagtctaatctcaaaccttttgagagagatatttcaactgaaatctatcaggccggtagcacaccttgtaatggtgttcaaggttttaattgttactttcctttacaatcatatggtttccaacccactaatggtgttggttaccaaccatacagagtagtagtactttcttttgaacttctacatgcaccagcaactgtttgtggacctaaaaagtctactaatttggttaaaaacaaatgtgtcaatttcgaagccgctgctaaggaagccgctgctaag

SEQ ID NO: 3 - DNA, 18 bp, Artificial Sequence
  linker sequence 1
ggctctggttctggctct

SEQ ID NO: 4 - DNA, 75 bp, Artificial Sequence
  linker sequence 2
gaagccgccgccaaggaagccgccgccaaggaagccgccgccaaggaagccgccgccaaggaagccgccgccaag

SEQ ID NO: 5 - DNA, 9 bp, Artificial Sequence
  linker sequence 3
tccggcggc

SEQ ID NO: 6 - DNA, 48 bp, Artificial Sequence
  signal peptide coding sequence
atgttcgtgttcctggtgctgctgcctctggtgtccagccagtgtgtg

SEQ ID NO: 7 - DNA, 753 bp, Artificial Sequence
  Seq.1
atgttcgtgttcctggtgctgctgcctctggtgtccagccagtgtgtgagagtccaaccaacagaatctattgttagatttcctaatattacaaacttgtgcccttttggtgaagtttttaacgccaccagatttgcatctgtttatgcttggaacaggaagagaatcagcaactgtgttgctgattattctgtcctatataattccgcatcattttccacttttaagtgttatggagtgtctcctactaaattaaatgatctctgctttactaatgtctatgcagattcatttgtaattagaggtgatgaagtcagacaaatcgctccagggcaaactggaaagattgctgattataattataaattaccagatgattttacaggctgcgttatagcttggaattctaacaatcttgattctaaggttggtggtaattataattaccggtatagattgtttaggaagtctaatctcaaaccttttgagagagatatttcaactgaaatctatcaggccggtagcacaccttgtaatggtgttcaaggttttaattgttactttcctttacaatcatatggtttccaacccactaatggtgttggttaccaaccatacagagtagtagtactttcttttgaacttctacatgcaccagcaactgtttgtggacctaaaaagtctactaatttggttaaaaacaaatgtgtcaatttcgaagccgctgctaaggaagccgctgctaagtgatga

SEQ ID NO: 8 - DNA, 834 bp, Artificial Sequence
  Seq.2
atgttcgtgttcctggtgctgctgcctctggtgtccagccagtgtgtgagagtccaaccaacagaatctattgttagatttcctaatattacaaacttgtgcccttttggtgaagtttttaacgccaccagatttgcatctgtttatgcttggaacaggaagagaatcagcaactgtgttgctgattattctgtcctatataattccgcatcattttccacttttaagtgttatggagtgtctcctactaaattaaatgatctctgctttactaatgtctatgcagattcatttgtaattagaggtgatgaagtcagacaaatcgctccagggcaaactggaaagattgctgattataattataaattaccagatgattttacaggctgcgttatagcttggaattctaacaatcttgattctaaggttggtggtaattataattaccggtatagattgtttaggaagtctaatctcaaaccttttgagagagatatttcaactgaaatctatcaggccggtagcacaccttgtaatggtgttcaaggttttaattgttactttcctttacaatcatatggtttccaacccactaatggtgttggttaccaaccatacagagtagtagtactttcttttgaacttctacatgcaccagcaactgtttgtggacctaaaaagtctactaatttggttaaaaacaaatgtgtcaatttcgaagccgctgctaaggaagccgctgctaagggctacatccctgaagcgcctagagacggccagtgctacgtgagatgcgacggcgaatgggtgctgctgtccactttcctgtgatga

SEQ ID NO: 9 - DNA, 852 bp, Artificial Sequence
  Seq.3
atgttcgtgttcctggtgctgctgcctctggtgtccagccagtgtgtgagagtccaaccaacagaatctattgttagatttcctaatattacaaacttgtgcccttttggtgaagtttttaacgccaccagatttgcatctgtttatgcttggaacaggaagagaatcagcaactgtgttgctgattattctgtcctatataattccgcatcattttccacttttaagtgttatggagtgtctcctactaaattaaatgatctctgctttactaatgtctatgcagattcatttgtaattagaggtgatgaagtcagacaaatcgctccagggcaaactggaaagattgctgattataattataaattaccagatgattttacaggctgcgttatagcttggaattctaacaatcttgattctaaggttggtggtaattataattaccggtatagattgtttaggaagtctaatctcaaaccttttgagagagatatttcaactgaaatctatcaggccggtagcacaccttgtaatggtgttcaaggttttaattgttactttcctttacaatcatatggtttccaacccactaatggtgttggttaccaaccatacagagtagtagtactttcttttgaacttctacatgcaccagcaactgtttgtggacctaaaaagtctactaatttggttaaaaacaaatgtgtcaatttcgaagccgctgctaaggaagccgctgctaagggctctggttctggctctggctacatccctgaagcgcctagagacggccagtgctacgtgagatgcgacggcgaatgggtgctgctgtccactttcctgtgatga

SEQ ID NO: 10 - DNA, 909 bp, Artificial Sequence
  Seq.4
atgttcgtgttcctggtgctgctgcctctggtgtccagccagtgtgtgagagtccaaccaacagaatctattgttagatttcctaatattacaaacttgtgcccttttggtgaagtttttaacgccaccagatttgcatctgtttatgcttggaacaggaagagaatcagcaactgtgttgctgattattctgtcctatataattccgcatcattttccacttttaagtgttatggagtgtctcctactaaattaaatgatctctgctttactaatgtctatgcagattcatttgtaattagaggtgatgaagtcagacaaatcgctccagggcaaactggaaagattgctgattataattataaattaccagatgattttacaggctgcgttatagcttggaattctaacaatcttgattctaaggttggtggtaattataattaccggtatagattgtttaggaagtctaatctcaaaccttttgagagagatatttcaactgaaatctatcaggccggtagcacaccttgtaatggtgttcaaggttttaattgttactttcctttacaatcatatggtttccaacccactaatggtgttggttaccaaccatacagagtagtagtactttcttttgaacttctacatgcaccagcaactgtttgtggacctaaaaagtctactaatttggttaaaaacaaatgtgtcaatttcgaagccgctgctaaggaagccgctgctaaggaagccgccgccaaggaagccgccgccaaggaagccgccgccaaggaagccgccgccaaggaagccgccgccaagggctacatccctgaagcgcctagagacggccagtgctacgtgagatgcgacggcgaatgggtgctgctgtccactttcctgtgatga

SEQ ID NO: 11 - DNA, 843 bp, Artificial Sequence
  Seq.5
atgttcgtgttcctggtgctgctgcctctggtgtccagccagtgtgtgagagtccaaccaacagaatctattgttagatttcctaatattacaaacttgtgcccttttggtgaagtttttaacgccaccagatttgcatctgtttatgcttggaacaggaagagaatcagcaactgtgttgctgattattctgtcctatataattccgcatcattttccacttttaagtgttatggagtgtctcctactaaattaaatgatctctgctttactaatgtctatgcagattcatttgtaattagaggtgatgaagtcagacaaatcgctccagggcaaactggaaagattgctgattataattataaattaccagatgattttacaggctgcgttatagcttggaattctaacaatcttgattctaaggttggtggtaattataattaccggtatagattgtttaggaagtctaatctcaaaccttttgagagagatatttcaactgaaatctatcaggccggtagcacaccttgtaatggtgttcaaggttttaattgttactttcctttacaatcatatggtttccaacccactaatggtgttggttaccaaccatacagagtagtagtactttcttttgaacttctacatgcaccagcaactgtttgtggacctaaaaagtctactaatttggttaaaaacaaatgtgtcaatttcgaagccgctgctaaggaagccgctgctaagtccggcggcggctacatccctgaagcgcctagagacggccagtgctacgtgagatgcgacggcgaatgggtgctgctgtccactttcctgtgatga

SEQ ID NO: 12 - DNA, 3825 bp, Artificial Sequence
  Seq.6
atgttcgtgttcctggtgctgctgcctctggtgtccagccagtgcgtgaatctgactactagaactcagctgcctcctgcgtacactaattccttcactagaggcgtgtactaccctgacaaagttttcagatcctccgttctgcactccactcaggacctgttcctgcctttcttctccaatgtgacttggttccacgcgatccacgtgtccggcactaatggcactaagagattcgacaatcctgtgctgcctttcaatgacggcgtgtacttcgcgtccactgaaaagtccaatatcatcagaggctggatcttcggcactactctggactccaagactcagtccctgctgatcgtgaataatgcgactaatgtggtgatcaaggtgtgcgaattccagttctgcaatgaccctttcctggacgtgtactaccacaagaataataagtcctggatgaagtccgaattcagagtgtactcctccgcgaataattgcactttcgaatacgtgtcccagcctttcctgatggacctggaaggcaagcagggcaatttcaagaatctgagagaattcgtgttcaagaatatcgatggttacttcaagatctactccaagcacactcctatcaatctggtgagagacctgcctcagggcttctccgcgctggaacctctggtggacctgccaatcggtatcaacatcactagattccagactctgctggcgctgcacagatcctacctgactcctggcgactcctcctccggctggactgcgggcgcggcggcgtactacgtgggctacctgcagcctagaactttcctgctgaagtacaatgaaaatggcactatcactgacgcggtggactgcgcgctggaccctctgtccgaaactaagtgcactctgaagtccttcactgtggaaaagggcatctaccagacttccaatttccgggtgcagcctaccgaaagcatcgtgcggttccccaatatcactaacctgtgccctttcggcgaagtgttcaatgccactcggttcgccagcgtgtacgcctggaaccggaagcggatctccaactgcgtggccgactactccgtgctgtacaattccgccagcttctccaccttcaagtgctacggcgtgagccctactaagctgaatgacctgtgcttcactaatgtgtacgccgacagcttcgtgatccggggcgacgaagtgcggcagatcgcccctggccagaccggcaagatcgccgactacaactacaagctgcccgacgacttcactggctgcgtgatcgcctggaattccaataatctggactccaaggtgggcggcaattacaattaccggtaccggctgttccggaagtccaatctgaagcctttcgaacgggacatctccaccgaaatctaccaggccggctccactccctgcaatggcgtgcagggcttcaattgctacttccctctgcagtcctacggcttccagcctactaatggcgtgggctaccagccttaccgggtggtggtgctgtccttcgaactgctgcacgcccctgccactgtgtgcggccctaagaagtccactaatctggtgaagaataagtgcgtgaatttcaatttcaatggcctgactggcactggcgtgctgactgaatccaataagaagttcctgcctttccagcagttcggccgggacatcgccgacactactgacgccgtgcgggaccctcagactctggaaatcctggacatcactccttgctccttcggcggcgtgtccgtgatcactcctggcactaatacttccaatcaggtggccgtgctgtaccagggcgtgaattgcactgaagtgcctgtggccatccacgccgaccagctgactcctacttggcgggtgtactccactggctccaatgtgttccagactcgggccggctgcctgatcggcgccgaacacgtgaataattcctacgaatgcgacatccctatcggcgccggcatctgcgcctcctaccagactcagactaattcccggcgggccgccgcctccgtggcctcccagtccatcatcgcctacactatgtccctgggcgccgaaaattccgtggcctactccaataattccatcgccatccctactaatttcactatctccgtgactactgaaatcctgcctgtgtccatgactaagacttccgtggactgcactatgtacatctgcggcgactccactgaatgctccaatctgctgctgcagtacggctccttctgcactcagctgaatcgggccctgactggcatcgccgtggaacaggacaagaatactcaggaagtgttcgcccaggtgaagcagatctacaagactcctcctatcaaggacttcggcggcttcaatttctcccagatcctgcctgacccttccaagccttccaagcggtccttcatcgaagacctgctgttcaataaggtgactctggccgacgccggcttcatcaagcagtacggcgactgcctgggcgacatcgccgcccgggacctgatctgcgcccagaagttcaatggcctgactgtgctgcctcctctgctgactgacgaaatgatcgcccagtacacttccgccctgctggccggcactatcacttccggctggactttcggcgccggcgccgccctgcagatccctttcgccatgcagatggcctaccggttcaatggcatcggcgtgactcagaatgtgctgtacgaaaatcagaagctgatcgccaatcagttcaattccgccatcggcaagatccaggactccctgtcctccactgcctccgccctgggcaagctgcaggacgtggtgaatcagaatgcccaggccctgaatactctggtgaagcagctgtcctccaatttcggcgccatctcctccgtgctgaatgacatcctgtcccggctggaccctcctgaagccgaagtgcagatcgaccggctgatcactggccggctgcagtccctgcagacttacgtgactcagcagctgatccgggccgccgaaatccgggcctccgccaatctggccgccactaagatgtccgaatgcgtgctgggccagtccaagcgggtggacttctgcggcaagggctaccacctgatgtccttccctcagtccgcccctcacggcgtggtgttcctgcacgtgacttacgtgcctgcccacgaaaagaatttcactactgcccctgccatctgccacgacggcaaggcccacttccctcgggaaggcgtgttcgtgtccaatggcactcactggttcgtgactcagcggaatttctacgaacctcagatcatcactactgacaatactttcgtgtccggcaattgcgacgtggtgatcggcatcgtgaataatactgtgtacgaccctctgcagcctgaactggactccttcaaggaagaactggacaagtacttcaagaatcacacttcccctgacgtggacctgggcgacatctccggcatcaatgcctccgtggtgaatatccagaaggaaatcgaccggctgaatgaagtggccaagaatctgaatgaatccctgatcgacctgcaggaactgggcaagtacgaacagtacatcaagtggccttggtacatctggctgggcttcatcgccggcctgatcgccatcgtgatggtgactatcatgctgtgctgcatgacttcctgctgctcctgcctgaagggctgctgctcctgcggctcctgctgcaagttcgacgaagacgactccgaacctgtgctgaagggcgtgaagctgcactacacttgatga